European Patent Specification EP 3 533 871 B1, published December 25, 2024. Title: Method for Evaluating Risk of Drug Hypersensitivity Reaction Induced by Sulfamethoxazole and/or Trimethoprim. Applicant: Chung Gung Memorial Hospital, Linkou. The sequence listing filed with the application follows.

SEQUENCE LISTING (3 sequences)

SEQ ID NO: 1 - DNA, 791 bp, Homo sapiens
gctcccactccatgaggtatttctacaccgccatgtcccggcccggccgcggggagccccgcttcatcaccgtgggctacgtggacgacacccagttcgtgaggttcgacagcgacgccacgagtccgaggatggcgccccgggcgccatggatagagcaggaggggccggagtattgggaccgggagacacagatctccaagaccaacacacagacttaccgagagaacctgcgcaccgcgctccgctactacaaccagagcgaggccggtgagtgaccccggcccggggcgcaggtcacgactccccatcccccacggacggcccgggtcgccccgagtctccgggtccgagatccgcctccctgaggccgcgggacccgcccagaccctcgaccggcgagagccccaggcgcgtttacccggtttcattttcagttgaggccaaaatccccgcgggttggtcggggcggggcggggctcgggggacggggctgaccgcggggccggggccagggtctcacatcatccagaggatgtatggctgcgacctggggccggacgggcgcctcctccgcgggcataaccagttagcctacgacggcaaggattacatcgccctgaacgaggacctgagctcctggaccgcggcggacaccgcggctcagatcacccagctcaagtgggaggcggcccgtgtggcggagcagctgagagcctacctggagggcgagtgcgtggagtggctccgcagatacctggagaacgggaaggagacgctgcagcgcgccc

SEQ ID NO: 2 - DNA, 19 bp, Artificial Sequence
  Primer
ggagccccgcttcatcacc

SEQ ID NO: 3 - DNA, 20 bp, Artificial Sequence
  Primer
tccttgccgtcgtaggctaa